European Patent Specification EP 3 385 368 B1, published March 1, 2023. Title: Method for producing mesenchymal stem cells. Applicant: TAKARA BIO INC. The sequence listing filed with the application follows.

SEQUENCE LISTING (9 sequences)

SEQ ID NO: 1 - protein, 87 aa, Artificial Sequence
  Partial region of fibronectin named III-8
PTDLRFTNIGPDTMRVTWAPPPSIDLTNFLVRYSPVKNEEDVAELSISPSDNAVVLTNLLPGTEYVVSVSSVYEQHESTPLRGRQKT

SEQ ID NO: 2 - protein, 90 aa, Artificial Sequence
  Partial region of fibronectin named III-9
GLDSPTGIDFSDITANSFTVHWIAPRATITGYRIRHHPEHFSGRPREDRVPHSRNSITLTNLTPGTEYVVSIVALNGREESPLLIGQQST

SEQ ID NO: 3 - protein, 94 aa, Artificial Sequence
  Partial region of fibronectin named III-10
VSDVPRDLEVVAATPTSLLISWDAPAVTVRYYRITYGETGGNSPVQEFTVPGSKSTATISGLKPGVDYTITVYAVTGRGDSPASSKPISINYRT

SEQ ID NO: 4 - protein, 84 aa, Artificial Sequence
  Partial region of fibronectin named III-11
QMQVTDVQDNSISVKWLPSSSPVTGYRVTTTPKNGPGPTKTKTAGPDQTEMTIEGLQPTVEYVVSVYAQNPSGESQPLVQTAVT

SEQ ID NO: 5 - protein, 92 aa, Artificial Sequence
  Partial region of fibronectin named III-12
AIPAPTDLKFTQVTPTSLSAQWTPPNVQLTGYRVRVTPKEKTGPMKEINLAPDSSSVVVSGLMVATKYEVSVYALKDTLTSRPAQGVVTTLE

SEQ ID NO: 6 - protein, 89 aa, Artificial Sequence
  Partial region of fibronectin named III-13
NVSPPRRARVTDATETTITISWRTKTETITGFQVDAVPANGQTPIQRTIKPDVRSYTITGLQPGTDYKIYLYTLNDNARSSPVVIDAST

SEQ ID NO: 7 - protein, 90 aa, Artificial Sequence
  Partial region of fibronectin named III-14
AIDAPSNLRFLATTPNSLLVSWQPPRARITGYIIKYEKPGSPPREVVPRPRPGVTEATITGLEPGTEYTIYVIALKNNQKSEPLIGRKKT

SEQ ID NO: 8 - protein, 25 aa, Artificial Sequence
  Partial region of fibronectin named CS-1
DELPQLVTLPHPNLHGPEILDVPST

SEQ ID NO: 9 - protein, 574 aa, Artificial Sequence
  Fibronectin fragment named Retronectin (CH-296)
PTDLRFTNIGPDTMRVTWAPPPSIDLTNFLVRYSPVKNEEDVAELSISPSDNAVVLTNLLPGTEYVVSVSSVYEQHESTPLRGRQKTGLDSPTGIDFSDITANSFTVHWIAPRATITGYRIRHHPEHFSGRPREDRVPHSRNSITLTNLTPGTEYVVSIVALNGREESPLLIGQQSTVSDVPRDLEVVAATPTSLLISWDAPAVTVRYYRITYGETGGNSPVQEFTVPGSKSTATISGLKPGVDYTITVYAVTGRGDSPASSKPISINYRTEIDKPSMAIPAPTDLKFTQVTPTSLSAQWTPPNVQLTGYRVRVTPKEKTGPMKEINLAPDSSSVVVSGLMVATKYEVSVYALKDTLTSRPAQGVVTTLENVSPPRRARVTDATETTITISWRTKTETITGFQVDAVPANGQTPIQRTIKPDVRSYTITGLQPGTDYKIYLYTLNDNARSSPVVIDASTAIDAPSNLRFLATTPNSLLVSWQPPRARITGYIIKYEKPGSPPREVVPRPRPGVTEATITGLEPGTEYTIYVIALKNNQKSEPLIGRKKTDELPQLVTLPHPNLHGPEILDVPST